European Patent Application EP 4 293 128 A2, published December 20, 2023. Title: DETECTING HEPATOCELLULAR CARCINOMA. Applicant: MAYO FOUNDATION FOR MEDICAL EDUCATION AND RESEARCH. The sequence listing filed with the application follows.

SEQUENCE LISTING (104 sequences)

SEQ ID NO: 1 - DNA, 17 bp, synthetic construct
  misc_feature 1..17: note = Synthetic
  source 1..17: mol_type = other DNA
gcgcgggaggattttcg

SEQ ID NO: 2 - DNA, 18 bp, synthetic construct
  misc_feature 1..18: note = Synthetic
  source 1..18: mol_type = other DNA
ccgccaccataaacgacc

SEQ ID NO: 3 - DNA, 21 bp, synthetic construct
  misc_feature 1..21: note = Synthetic
  source 1..21: mol_type = other DNA
ccacggacgcgaaatcgaaat

SEQ ID NO: 4 - DNA, 21 bp, synthetic construct
  misc_feature 1..21: note = Synthetic
  source 1..21: mol_type = other DNA
cgttcgttacgtcgttttcgt

SEQ ID NO: 5 - DNA, 17 bp, synthetic construct
  misc_feature 1..17: note = Synthetic
  source 1..17: mol_type = other DNA
gatcgacgcgactcgac

SEQ ID NO: 6 - DNA, 21 bp, synthetic construct
  misc_feature 1..21: note = Synthetic
  source 1..21: mol_type = other DNA
ccacggacgctcgacgtcgcc

SEQ ID NO: 7 - DNA, 17 bp, synthetic construct
  misc_feature 1..17: note = Synthetic
  source 1..17: mol_type = other DNA
gcgggagtttggcgtag

SEQ ID NO: 8 - DNA, 21 bp, synthetic construct
  misc_feature 1..21: note = Synthetic
  source 1..21: mol_type = other DNA
cgcgcaaataccgaataaacg

SEQ ID NO: 9 - DNA, 21 bp, synthetic construct
  misc_feature 1..21: note = Synthetic
  source 1..21: mol_type = other DNA
ccacggacggtcggtagatcg

SEQ ID NO: 10 - DNA, 18 bp, synthetic construct
  misc_feature 1..18: note = Synthetic
  source 1..18: mol_type = other DNA
gcgcgttgtttcgtttcg

SEQ ID NO: 11 - DNA, 20 bp, synthetic construct
  misc_feature 1..20: note = Synthetic
  source 1..20: mol_type = other DNA
cgtcacctaccgcaaatacg

SEQ ID NO: 12 - DNA, 21 bp, synthetic construct
  misc_feature 1..21: note = Synthetic
  source 1..21: mol_type = other DNA
ccacggacggcggataaggag

SEQ ID NO: 13 - DNA, 19 bp, synthetic construct
  misc_feature 1..19: note = Synthetic
  source 1..19: mol_type = other DNA
agtacgtaagtagagcgcg

SEQ ID NO: 14 - DNA, 22 bp, synthetic construct
  misc_feature 1..22: note = Synthetic
  source 1..22: mol_type = other DNA
ctaaaattaactacgccgccgt

SEQ ID NO: 15 - DNA, 21 bp, synthetic construct
  misc_feature 1..21: note = Synthetic
  source 1..21: mol_type = other DNA
ccacggacggagaacgttcga

SEQ ID NO: 16 - DNA, 21 bp, synthetic construct
  misc_feature 1..21: note = Synthetic
  source 1..21: mol_type = other DNA
ggcgtcgcgttttttagagaa

SEQ ID NO: 17 - DNA, 28 bp, synthetic construct
  misc_feature 1..28: note = Synthetic
  source 1..28: mol_type = other DNA
ttccttttcgttcgtataaaatttcgtt

SEQ ID NO: 18 - DNA, 21 bp, synthetic construct
  misc_feature 1..21: note = Synthetic
  source 1..21: mol_type = other DNA
ccacggacgatcgggttttag

SEQ ID NO: 19 - DNA, 17 bp, synthetic construct
  misc_feature 1..17: note = Synthetic
  source 1..17: mol_type = other DNA
tgcgtatggtgggcgag

SEQ ID NO: 20 - DNA, 26 bp, synthetic construct
  misc_feature 1..26: note = Synthetic
  source 1..26: mol_type = other DNA
cctaatttacacgtcaaccaatcgaa

SEQ ID NO: 21 - DNA, 21 bp, synthetic construct
  misc_feature 1..21: note = Synthetic
  source 1..21: mol_type = other DNA
ccacggacggcgcgtgcgttt

SEQ ID NO: 22 - DNA, 27 bp, synthetic construct
  misc_feature 1..27: note = Synthetic
  source 1..27: mol_type = other DNA
tttgtttttttgattaggtgtttaaga

SEQ ID NO: 23 - DNA, 21 bp, synthetic construct
  misc_feature 1..21: note = Synthetic
  source 1..21: mol_type = other DNA
caccaacctcataaccttatc

SEQ ID NO: 24 - DNA, 21 bp, synthetic construct
  misc_feature 1..21: note = Synthetic
  source 1..21: mol_type = other DNA
gacgcggagatagtgttgtgg

SEQ ID NO: 25 - DNA, 22 bp, synthetic construct
  misc_feature 1..22: note = Synthetic
  source 1..22: mol_type = other DNA
gcgttttagttagatagggcgg

SEQ ID NO: 26 - DNA, 20 bp, synthetic construct
  misc_feature 1..20: note = Synthetic
  source 1..20: mol_type = other DNA
gaaaaccccttccccgaaac

SEQ ID NO: 27 - DNA, 20 bp, synthetic construct
  misc_feature 1..20: note = Synthetic
  source 1..20: mol_type = other DNA
cgccgaggcgcacgcctaaa

SEQ ID NO: 28 - DNA, 26 bp, synthetic construct
  misc_feature 1..26: note = Synthetic
  source 1..26: mol_type = other DNA
agtcgtttttttaggtagtttaggcg

SEQ ID NO: 29 - DNA, 19 bp, synthetic construct
  misc_feature 1..19: note = Synthetic
  source 1..19: mol_type = other DNA
cgacctttacaatcgccgc

SEQ ID NO: 30 - DNA, 20 bp, synthetic construct
  misc_feature 1..20: note = Synthetic
  source 1..20: mol_type = other DNA
cgccgaggggcggtagttgt

SEQ ID NO: 31 - DNA, 16 bp, synthetic construct
  misc_feature 1..16: note = Synthetic
  source 1..16: mol_type = other DNA
gggagcggtcgcgtag

SEQ ID NO: 32 - DNA, 28 bp, synthetic construct
  misc_feature 1..28: note = Synthetic
  source 1..28: mol_type = other DNA
gcacctaactaaacaaaacgaactaaac

SEQ ID NO: 33 - DNA, 20 bp, synthetic construct
  misc_feature 1..20: note = Synthetic
  source 1..20: mol_type = other DNA
cgccgaggcgcaaacgcaaa

SEQ ID NO: 34 - DNA, 17 bp, synthetic construct
  misc_feature 1..17: note = Synthetic
  source 1..17: mol_type = other DNA
aggtggcgcgtattacg

SEQ ID NO: 35 - DNA, 20 bp, synthetic construct
  misc_feature 1..20: note = Synthetic
  source 1..20: mol_type = other DNA
cctactaaacgcgctcaacc

SEQ ID NO: 36 - DNA, 20 bp, synthetic construct
  misc_feature 1..20: note = Synthetic
  source 1..20: mol_type = other DNA
cgccgaggcgctcgattccc

SEQ ID NO: 37 - DNA, 19 bp, synthetic construct
  misc_feature 1..19: note = Synthetic
  source 1..19: mol_type = other DNA
ttcgatattgggtgtcgcg

SEQ ID NO: 38 - DNA, 21 bp, synthetic construct
  misc_feature 1..21: note = Synthetic
  source 1..21: mol_type = other DNA
cgcgaaaaccaaaaacgaaac

SEQ ID NO: 39 - DNA, 20 bp, synthetic construct
  misc_feature 1..20: note = Synthetic
  source 1..20: mol_type = other DNA
cgccgagggaggcggggttc

SEQ ID NO: 40 - DNA, 19 bp, synthetic construct
  misc_feature 1..19: note = Synthetic
  source 1..19: mol_type = other DNA
gcgttaatttcgcgaggta

SEQ ID NO: 41 - DNA, 28 bp, synthetic construct
  misc_feature 1..28: note = Synthetic
  source 1..28: mol_type = other DNA
acaatactcttatatattaacgccgctc

SEQ ID NO: 42 - DNA, 20 bp, synthetic construct
  misc_feature 1..20: note = Synthetic
  source 1..20: mol_type = other DNA
cgccgaggaggcgacggagg

SEQ ID NO: 43 - DNA, 19 bp, synthetic construct
  misc_feature 1..19: note = Synthetic
  source 1..19: mol_type = other DNA
tttgtttcggtttttggcg

SEQ ID NO: 44 - DNA, 21 bp, synthetic construct
  misc_feature 1..21: note = Synthetic
  source 1..21: mol_type = other DNA
accataaacgaccgaaatcga

SEQ ID NO: 45 - DNA, 21 bp, synthetic construct
  misc_feature 1..21: note = Synthetic
  source 1..21: mol_type = other DNA
ccacggacggcgggaggattt

SEQ ID NO: 46 - DNA, 21 bp, synthetic construct
  misc_feature 1..21: note = Synthetic
  source 1..21: mol_type = other DNA
cgttcgttacgtcgttttcgt

SEQ ID NO: 47 - DNA, 17 bp, synthetic construct
  misc_feature 1..17: note = Synthetic
  source 1..17: mol_type = other DNA
gatcgacgcgactcgac

SEQ ID NO: 48 - DNA, 21 bp, synthetic construct
  misc_feature 1..21: note = Synthetic
  source 1..21: mol_type = other DNA
ccacggacgctcgacgtcgcc

SEQ ID NO: 49 - DNA, 22 bp, synthetic construct
  misc_feature 1..22: note = Synthetic
  source 1..22: mol_type = other DNA
gcgttttagttagatagggcgg

SEQ ID NO: 50 - DNA, 20 bp, synthetic construct
  misc_feature 1..20: note = Synthetic
  source 1..20: mol_type = other DNA
gaaaaccccttccccgaaac

SEQ ID NO: 51 - DNA, 20 bp, synthetic construct
  misc_feature 1..20: note = Synthetic
  source 1..20: mol_type = other DNA
cgccgaggcgcacgcctaaa

SEQ ID NO: 52 - DNA, 17 bp, synthetic construct
  misc_feature 1..17: note = Synthetic
  source 1..17: mol_type = other DNA
gcgggagtttggcgtag

SEQ ID NO: 53 - DNA, 21 bp, synthetic construct
  misc_feature 1..21: note = Synthetic
  source 1..21: mol_type = other DNA
cgcgcaaataccgaataaacg

SEQ ID NO: 54 - DNA, 21 bp, synthetic construct
  misc_feature 1..21: note = Synthetic
  source 1..21: mol_type = other DNA
ccacggacggtcggtagatcg

SEQ ID NO: 55 - DNA, 16 bp, synthetic construct
  misc_feature 1..16: note = Synthetic
  source 1..16: mol_type = other DNA
gggagcggtcgcgtag

SEQ ID NO: 56 - DNA, 28 bp, synthetic construct
  misc_feature 1..28: note = Synthetic
  source 1..28: mol_type = other DNA
gcacctaactaaacaaaacgaactaaac

SEQ ID NO: 57 - DNA, 20 bp, synthetic construct
  misc_feature 1..20: note = Synthetic
  source 1..20: mol_type = other DNA
cgccgaggcgcaaacgcaaa

SEQ ID NO: 58 - DNA, 18 bp, synthetic construct
  misc_feature 1..18: note = Synthetic
  source 1..18: mol_type = other DNA
gcgcgttgtttcgtttcg

SEQ ID NO: 59 - DNA, 20 bp, synthetic construct
  misc_feature 1..20: note = Synthetic
  source 1..20: mol_type = other DNA
cgtcacctaccgcaaatacg

SEQ ID NO: 60 - DNA, 21 bp, synthetic construct
  misc_feature 1..21: note = Synthetic
  source 1..21: mol_type = other DNA
ccacggacggcggataaggag

SEQ ID NO: 61 - DNA, 19 bp, synthetic construct
  misc_feature 1..19: note = Synthetic
  source 1..19: mol_type = other DNA
agtacgtaagtagagcgcg

SEQ ID NO: 62 - DNA, 22 bp, synthetic construct
  misc_feature 1..22: note = Synthetic
  source 1..22: mol_type = other DNA
ctaaaattaactacgccgccgt

SEQ ID NO: 63 - DNA, 21 bp, synthetic construct
  misc_feature 1..21: note = Synthetic
  source 1..21: mol_type = other DNA
ccacggacggagaacgttcga

SEQ ID NO: 64 - DNA, 24 bp, synthetic construct
  misc_feature 1..24: note = Synthetic
  source 1..24: mol_type = other DNA
cgttcgttcgttattttttttcga

SEQ ID NO: 65 - DNA, 19 bp, synthetic construct
  misc_feature 1..19: note = Synthetic
  source 1..19: mol_type = other DNA
gcccgcgaaaaccaaaaac

SEQ ID NO: 66 - DNA, 20 bp, synthetic construct
  misc_feature 1..20: note = Synthetic
  source 1..20: mol_type = other DNA
cgccgaggcgaaactcacct

SEQ ID NO: 67 - DNA, 22 bp, synthetic construct
  misc_feature 1..22: note = Synthetic
  source 1..22: mol_type = other DNA
gcgtttttttttagcggggtta

SEQ ID NO: 68 - DNA, 21 bp, synthetic construct
  misc_feature 1..21: note = Synthetic
  source 1..21: mol_type = other DNA
ccgaaactaaaattctcccgc

SEQ ID NO: 69 - DNA, 20 bp, synthetic construct
  misc_feature 1..20: note = Synthetic
  source 1..20: mol_type = other DNA
cgccgaggatgagcgtgtta

SEQ ID NO: 70 - DNA, 19 bp, synthetic construct
  misc_feature 1..19: note = Synthetic
  source 1..19: mol_type = other DNA
cggttttcgtttgggtacg

SEQ ID NO: 71 - DNA, 17 bp, synthetic construct
  misc_feature 1..17: note = Synthetic
  source 1..17: mol_type = other DNA
ccaacccaaaccacgcc

SEQ ID NO: 72 - DNA, 21 bp, synthetic construct
  misc_feature 1..21: note = Synthetic
  source 1..21: mol_type = other DNA
ccacggacgcgcgccgtacga

SEQ ID NO: 73 - DNA, 16 bp, synthetic construct
  misc_feature 1..16: note = Synthetic
  source 1..16: mol_type = other DNA
ggaggttggcggggag

SEQ ID NO: 74 - DNA, 23 bp, synthetic construct
  misc_feature 1..23: note = Synthetic
  source 1..23: mol_type = other DNA
catatactatcgccttccgactc

SEQ ID NO: 75 - DNA, 20 bp, synthetic construct
  misc_feature 1..20: note = Synthetic
  source 1..20: mol_type = other DNA
cgccgaggcgtaacaaaaac

SEQ ID NO: 76 - DNA, 19 bp, synthetic construct
  misc_feature 1..19: note = Synthetic
  source 1..19: mol_type = other DNA
tcgttttaggtgagtcgcg

SEQ ID NO: 77 - DNA, 24 bp, synthetic construct
  misc_feature 1..24: note = Synthetic
  source 1..24: mol_type = other DNA
aaataaaaccgccgaaaaaacaac

SEQ ID NO: 78 - DNA, 21 bp, synthetic construct
  misc_feature 1..21: note = Synthetic
  source 1..21: mol_type = other DNA
ccacggacgcgctacaaacgc

SEQ ID NO: 79 - DNA, 17 bp, synthetic construct
  misc_feature 1..17: note = Synthetic
  source 1..17: mol_type = other DNA
ggaggggtttcgttcgt

SEQ ID NO: 80 - DNA, 29 bp, synthetic construct
  misc_feature 1..29: note = Synthetic
  source 1..29: mol_type = other DNA
ctactatcgacgctaaaaataaaacgaac

SEQ ID NO: 81 - DNA, 20 bp, synthetic construct
  misc_feature 1..20: note = Synthetic
  source 1..20: mol_type = other DNA
cgccgaggcgcgacctaaaa

SEQ ID NO: 82 - DNA, 17 bp, synthetic construct
  misc_feature 1..17: note = Synthetic
  source 1..17: mol_type = other DNA
aggtggcgcgtattacg

SEQ ID NO: 83 - DNA, 20 bp, synthetic construct
  misc_feature 1..20: note = Synthetic
  source 1..20: mol_type = other DNA
cctactaaacgcgctcaacc

SEQ ID NO: 84 - DNA, 20 bp, synthetic construct
  misc_feature 1..20: note = Synthetic
  source 1..20: mol_type = other DNA
cgccgaggcgctcgattccc

SEQ ID NO: 85 - DNA, 19 bp, synthetic construct
  misc_feature 1..19: note = Synthetic
  source 1..19: mol_type = other DNA
gcgttaatttcgcgaggta

SEQ ID NO: 86 - DNA, 28 bp, synthetic construct
  misc_feature 1..28: note = Synthetic
  source 1..28: mol_type = other DNA
acaatactcttatatattaacgccgctc

SEQ ID NO: 87 - DNA, 20 bp, synthetic construct
  misc_feature 1..20: note = Synthetic
  source 1..20: mol_type = other DNA
cgccgaggaggcgacggagg

SEQ ID NO: 88 - DNA, 26 bp, synthetic construct
  misc_feature 1..26: note = Synthetic
  source 1..26: mol_type = other DNA
agtcgtttttttaggtagtttaggcg

SEQ ID NO: 89 - DNA, 19 bp, synthetic construct
  misc_feature 1..19: note = Synthetic
  source 1..19: mol_type = other DNA
cgacctttacaatcgccgc

SEQ ID NO: 90 - DNA, 20 bp, synthetic construct
  misc_feature 1..20: note = Synthetic
  source 1..20: mol_type = other DNA
cgccgaggggcggtagttgt

SEQ ID NO: 91 - DNA, 21 bp, synthetic construct
  misc_feature 1..21: note = Synthetic
  source 1..21: mol_type = other DNA
ggcgtcgcgttttttagagaa

SEQ ID NO: 92 - DNA, 27 bp, synthetic construct
  misc_feature 1..27: note = Synthetic
  source 1..27: mol_type = other DNA
ttccttttcgttcgtataaaatttcgt

SEQ ID NO: 93 - DNA, 21 bp, synthetic construct
  misc_feature 1..21: note = Synthetic
  source 1..21: mol_type = other DNA
ccacggacgatcgggttttag

SEQ ID NO: 94 - DNA, 20 bp, synthetic construct
  misc_feature 1..20: note = Synthetic
  source 1..20: mol_type = other DNA
cgccgaggatcgggttttag

SEQ ID NO: 95 - DNA, 29 bp, synthetic construct
  misc_feature 1..29: note = Synthetic
  source 1..29: mol_type = other DNA
agccggttttccggctgagactccgcgtc

SEQ ID NO: 96 - DNA, 32 bp, synthetic construct
  misc_feature 1..32: note = Synthetic
  misc_feature 3: note = modified with quencher
  source 1..32: mol_type = other DNA
tctagccggttttccggctgagactccgcgtc

SEQ ID NO: 97 - DNA, 29 bp, synthetic construct
  misc_feature 1..29: note = Synthetic
  source 1..29: mol_type = other DNA
agccggttttccggctgagacgtccgtgg

SEQ ID NO: 98 - DNA, 31 bp, synthetic construct
  misc_feature 1..31: note = Synthetic
  misc_feature 3: note = modified with quencher
  source 1..31: mol_type = other DNA
tctagccgttttccggctgagacgtccgtgg

SEQ ID NO: 99 - DNA, 28 bp, synthetic construct
  misc_feature 1..28: note = Synthetic
  source 1..28: mol_type = other DNA
agccggttttccggctgagacctcggcg

SEQ ID NO: 100 - DNA, 31 bp, synthetic construct
  misc_feature 1..31: note = Synthetic
  misc_feature 3: note = modified with quencher
  source 1..31: mol_type = other DNA
tctagccggttttccggctgagacctcggcg

SEQ ID NO: 101-104 - skipped (4 entries)